European Patent Application EP 4 725 955 A1, published April 15, 2026. Title: 靶向c-Met的肽、包含所述肽的药物组合物及其用途. Applicant: 南京安吉生物科技有限公司. The sequence listing filed with the application follows.

SEQUENCE LISTING (150 sequences)

SEQ ID NO: 1 - protein, 7 aa, synthetic construct
RSPYANS

SEQ ID NO: 2 - protein, 7 aa, synthetic construct
DQIIANN

SEQ ID NO: 3 - protein, 7 aa, synthetic construct
AQIIANN

SEQ ID NO: 4 - protein, 7 aa, synthetic construct
DAIIANN

SEQ ID NO: 5 - protein, 7 aa, synthetic construct
DQAIANN

SEQ ID NO: 6 - protein, 7 aa, synthetic construct
DQIAANN

SEQ ID NO: 7 - protein, 7 aa, synthetic construct
DQIIAAN

SEQ ID NO: 8 - protein, 7 aa, synthetic construct
DQIIANA

SEQ ID NO: 9 - protein, 7 aa, synthetic construct
HQIIANN

SEQ ID NO: 10 - protein, 7 aa, synthetic construct
RQIIANN

SEQ ID NO: 11 - protein, 7 aa, synthetic construct
FQIIANN

SEQ ID NO: 12 - protein, 7 aa, synthetic construct
AQIIANN

SEQ ID NO: 13 - protein, 7 aa, synthetic construct
CQIIANN

SEQ ID NO: 14 - protein, 7 aa, synthetic construct
GQIIANN

SEQ ID NO: 15 - protein, 7 aa, synthetic construct
QQIIANN

SEQ ID NO: 16 - protein, 7 aa, synthetic construct
EQIIANN

SEQ ID NO: 17 - protein, 7 aa, synthetic construct
KQIIANN

SEQ ID NO: 18 - protein, 7 aa, synthetic construct
LQIIANN

SEQ ID NO: 19 - protein, 7 aa, synthetic construct
MQIIANN

SEQ ID NO: 20 - protein, 7 aa, synthetic construct
NQIIANN

SEQ ID NO: 21 - protein, 7 aa, synthetic construct
SQIIANN

SEQ ID NO: 22 - protein, 7 aa, synthetic construct
YQIIANN

SEQ ID NO: 23 - protein, 7 aa, synthetic construct
TQIIANN

SEQ ID NO: 24 - protein, 7 aa, synthetic construct
IQIIANN

SEQ ID NO: 25 - protein, 7 aa, synthetic construct
WQIIANN

SEQ ID NO: 26 - protein, 7 aa, synthetic construct
PQIIANN

SEQ ID NO: 27 - protein, 7 aa, synthetic construct
VQIIANN

SEQ ID NO: 28 - protein, 7 aa, synthetic construct
RHIIANN

SEQ ID NO: 29 - protein, 7 aa, synthetic construct
RDIIANN

SEQ ID NO: 30 - protein, 7 aa, synthetic construct
RRIIANN

SEQ ID NO: 31 - protein, 7 aa, synthetic construct
RFIIANN

SEQ ID NO: 32 - protein, 7 aa, synthetic construct
RAIIANN

SEQ ID NO: 33 - protein, 7 aa, synthetic construct
RCIIANN

SEQ ID NO: 34 - protein, 7 aa, synthetic construct
RGIIANN

SEQ ID NO: 35 - protein, 7 aa, synthetic construct
REIIANN

SEQ ID NO: 36 - protein, 7 aa, synthetic construct
RKIIANN

SEQ ID NO: 37 - protein, 7 aa, synthetic construct
RLIIANN

SEQ ID NO: 38 - protein, 7 aa, synthetic construct
RMIIANN

SEQ ID NO: 39 - protein, 7 aa, synthetic construct
RNIIANN

SEQ ID NO: 40 - protein, 7 aa, synthetic construct
RSIIANN

SEQ ID NO: 41 - protein, 7 aa, synthetic construct
RYIIANN

SEQ ID NO: 42 - protein, 7 aa, synthetic construct
RTIIANN

SEQ ID NO: 43 - protein, 7 aa, synthetic construct
RIIIANN

SEQ ID NO: 44 - protein, 7 aa, synthetic construct
RWIIANN

SEQ ID NO: 45 - protein, 7 aa, synthetic construct
RPIIANN

SEQ ID NO: 46 - protein, 7 aa, synthetic construct
RVIIANN

SEQ ID NO: 47 - protein, 7 aa, synthetic construct
RSHIANN

SEQ ID NO: 48 - protein, 7 aa, synthetic construct
RSDIANN

SEQ ID NO: 49 - protein, 7 aa, synthetic construct
RSRIANN

SEQ ID NO: 50 - protein, 7 aa, synthetic construct
RSFIANN

SEQ ID NO: 51 - protein, 7 aa, synthetic construct
RSAIANN

SEQ ID NO: 52 - protein, 7 aa, synthetic construct
RSCIANN

SEQ ID NO: 53 - protein, 7 aa, synthetic construct
RSGIANN

SEQ ID NO: 54 - protein, 7 aa, synthetic construct
RSQIANN

SEQ ID NO: 55 - protein, 7 aa, synthetic construct
RSEIANN

SEQ ID NO: 56 - protein, 7 aa, synthetic construct
RSKIANN

SEQ ID NO: 57 - protein, 7 aa, synthetic construct
RSLIANN

SEQ ID NO: 58 - protein, 7 aa, synthetic construct
RSMIANN

SEQ ID NO: 59 - protein, 7 aa, synthetic construct
RSNIANN

SEQ ID NO: 60 - protein, 7 aa, synthetic construct
RSSIANN

SEQ ID NO: 61 - protein, 7 aa, synthetic construct
RSYIANN

SEQ ID NO: 62 - protein, 7 aa, synthetic construct
RSTIANN

SEQ ID NO: 63 - protein, 7 aa, synthetic construct
RSWIANN

SEQ ID NO: 64 - protein, 7 aa, synthetic construct
RSPIANN

SEQ ID NO: 65 - protein, 7 aa, synthetic construct
RSVIANN

SEQ ID NO: 66 - protein, 7 aa, synthetic construct
RSPHANN

SEQ ID NO: 67 - protein, 7 aa, synthetic construct
RSPDANN

SEQ ID NO: 68 - protein, 7 aa, synthetic construct
RSPRANN

SEQ ID NO: 69 - protein, 7 aa, synthetic construct
RSPFANN

SEQ ID NO: 70 - protein, 7 aa, synthetic construct
RSPAANN

SEQ ID NO: 71 - protein, 7 aa, synthetic construct
RSPCANN

SEQ ID NO: 72 - protein, 7 aa, synthetic construct
RSPGANN

SEQ ID NO: 73 - protein, 7 aa, synthetic construct
RSPQANN

SEQ ID NO: 74 - protein, 7 aa, synthetic construct
RSPEANN

SEQ ID NO: 75 - protein, 7 aa, synthetic construct
RSPKANN

SEQ ID NO: 76 - protein, 7 aa, synthetic construct
RSPLANN

SEQ ID NO: 77 - protein, 7 aa, synthetic construct
RSPMANN

SEQ ID NO: 78 - protein, 7 aa, synthetic construct
RSPNANN

SEQ ID NO: 79 - protein, 7 aa, synthetic construct
RSPSANN

SEQ ID NO: 80 - protein, 7 aa, synthetic construct
RSPYANN

SEQ ID NO: 81 - protein, 7 aa, synthetic construct
RSPTANN

SEQ ID NO: 82 - protein, 7 aa, synthetic construct
RSPWANN

SEQ ID NO: 83 - protein, 7 aa, synthetic construct
RSPPANN

SEQ ID NO: 84 - protein, 7 aa, synthetic construct
RSPVANN

SEQ ID NO: 85 - protein, 7 aa, synthetic construct
RSPYANN

SEQ ID NO: 86 - protein, 7 aa, synthetic construct
RSPYHNN

SEQ ID NO: 87 - protein, 7 aa, synthetic construct
RSPYDNN

SEQ ID NO: 88 - protein, 7 aa, synthetic construct
RSPYRNN

SEQ ID NO: 89 - protein, 7 aa, synthetic construct
RSPYFNN

SEQ ID NO: 90 - protein, 7 aa, synthetic construct
RSPYCNN

SEQ ID NO: 91 - protein, 7 aa, synthetic construct
RSPYGNN

SEQ ID NO: 92 - protein, 7 aa, synthetic construct
RSPYQNN

SEQ ID NO: 93 - protein, 7 aa, synthetic construct
RSPYENN

SEQ ID NO: 94 - protein, 7 aa, synthetic construct
RSPYKNN

SEQ ID NO: 95 - protein, 7 aa, synthetic construct
RSPYLNN

SEQ ID NO: 96 - protein, 7 aa, synthetic construct
RSPYMNN

SEQ ID NO: 97 - protein, 7 aa, synthetic construct
RSPYNNN

SEQ ID NO: 98 - protein, 7 aa, synthetic construct
RSPYSNN

SEQ ID NO: 99 - protein, 7 aa, synthetic construct
RSPYYNN

SEQ ID NO: 100 - protein, 7 aa, synthetic construct
RSPYTNN

SEQ ID NO: 101 - protein, 7 aa, synthetic construct
RSPYINN

SEQ ID NO: 102 - protein, 7 aa, synthetic construct
RSPYWNN

SEQ ID NO: 103 - protein, 7 aa, synthetic construct
RSPYPNN

SEQ ID NO: 104 - protein, 7 aa, synthetic construct
RSPYVNN

SEQ ID NO: 105 - protein, 7 aa, synthetic construct
RSPYANN

SEQ ID NO: 106 - protein, 7 aa, synthetic construct
RSPYAHN

SEQ ID NO: 107 - protein, 7 aa, synthetic construct
RSPYADN

SEQ ID NO: 108 - protein, 7 aa, synthetic construct
RSPYARN

SEQ ID NO: 109 - protein, 7 aa, synthetic construct
RSPYAFN

SEQ ID NO: 110 - protein, 7 aa, synthetic construct
RSPYAAN

SEQ ID NO: 111 - protein, 7 aa, synthetic construct
RSPYACN

SEQ ID NO: 112 - protein, 7 aa, synthetic construct
RSPYAGN

SEQ ID NO: 113 - protein, 7 aa, synthetic construct
RSPYAQN

SEQ ID NO: 114 - protein, 7 aa, synthetic construct
RSPYAEN

SEQ ID NO: 115 - protein, 7 aa, synthetic construct
RSPYAKN

SEQ ID NO: 116 - protein, 7 aa, synthetic construct
RSPYALN

SEQ ID NO: 117 - protein, 7 aa, synthetic construct
RSPYAMN

SEQ ID NO: 118 - protein, 7 aa, synthetic construct
RSPYASN

SEQ ID NO: 119 - protein, 7 aa, synthetic construct
RSPYAYN

SEQ ID NO: 120 - protein, 7 aa, synthetic construct
RSPYATN

SEQ ID NO: 121 - protein, 7 aa, synthetic construct
RSPYAIN

SEQ ID NO: 122 - protein, 7 aa, synthetic construct
RSPYAWN

SEQ ID NO: 123 - protein, 7 aa, synthetic construct
RSPYAPN

SEQ ID NO: 124 - protein, 7 aa, synthetic construct
RSPYAVN

SEQ ID NO: 125 - protein, 7 aa, synthetic construct
RSPYANN

SEQ ID NO: 126 - protein, 7 aa, synthetic construct
RSPYANH

SEQ ID NO: 127 - protein, 7 aa, synthetic construct
RSPYAND

SEQ ID NO: 128 - protein, 7 aa, synthetic construct
RSPYANR

SEQ ID NO: 129 - protein, 7 aa, synthetic construct
RSPYANF

SEQ ID NO: 130 - protein, 7 aa, synthetic construct
RSPYANA

SEQ ID NO: 131 - protein, 7 aa, synthetic construct
RSPYANC

SEQ ID NO: 132 - protein, 7 aa, synthetic construct
RSPYANG

SEQ ID NO: 133 - protein, 7 aa, synthetic construct
RSPYANQ

SEQ ID NO: 134 - protein, 7 aa, synthetic construct
RSPYANE

SEQ ID NO: 135 - protein, 7 aa, synthetic construct
RSPYANK

SEQ ID NO: 136 - protein, 7 aa, synthetic construct
RSPYANL

SEQ ID NO: 137 - protein, 7 aa, synthetic construct
RSPYANM

SEQ ID NO: 138 - protein, 7 aa, synthetic construct
RSPYANY

SEQ ID NO: 139 - protein, 7 aa, synthetic construct
RSPYANT

SEQ ID NO: 140 - protein, 7 aa, synthetic construct
RSPYANI

SEQ ID NO: 141 - protein, 7 aa, synthetic construct
RSPYANW

SEQ ID NO: 142 - protein, 7 aa, synthetic construct
RSPYANP

SEQ ID NO: 143 - protein, 7 aa, synthetic construct
RSPYANV

SEQ ID NO: 144 - protein, 7 aa, synthetic construct
RSPYCNS

SEQ ID NO: 145 - protein, 7 aa, synthetic construct
ASPYANS

SEQ ID NO: 146 - protein, 7 aa, synthetic construct
RAPYANS

SEQ ID NO: 147 - protein, 7 aa, synthetic construct
RSAYANS

SEQ ID NO: 148 - protein, 7 aa, synthetic construct
RSPAANS

SEQ ID NO: 149 - protein, 7 aa, synthetic construct
RSPYAAS

SEQ ID NO: 150 - protein, 7 aa, synthetic construct
RSPYANA